European Patent Application EP 4 306 124 A1, published January 17, 2024. Title: A composition for preventing or treating degenerative brain diseases. Applicant: KOLON LIFE SCIENCE, INC. The sequence listing filed with the application follows.

SEQUENCE LISTING (16 sequences)

SEQ ID NO: 1 - protein, 178 aa, Homo sapiens
MHSSALLCCLVLLTGVRASPGQGTQSENSCTHFPGNLPNMLRDLRDAFSRVKTFFQMKDQLDNLLLKESLLEDFKGYLGCQALSEMIQFYLEEVMPQAENQDPDIKAHVNSLGENLKTLRLRLRRCHRFLPCENKSKAVEQVKNAFNKLQEKGIYKAMSEFDIFINYIEAYMTMKIRN

SEQ ID NO: 2 - DNA, 1600 bp, Homo sapiens
aaaccacaagacagacttgcaaaagaaggcatgcacagctcagcactgctctgttgcctggtcctcctgactggggtgagggccagcccaggccagggcacccagtctgagaacagctgcacccacttcccaggcaacctgcctaacatgcttcgagatctccgagatgccttcagcagagtgaagactttctttcaaatgaaggatcagctggacaacttgttgttaaaggagtccttgctggaggactttaagggttacctgggttgccaagccttgtctgagatgatccagttttacctggaggaggtgatgccccaagctgagaaccaagacccagacatcaaggcgcatgtgaactccctgggggagaacctgaagaccctcaggctgaggctacggcgctgtcatcgatttcttccctgtgaaaacaagagcaaggccgtggagcaggtgaagaatgcctttaataagctccaagagaaaggcatctacaaagccatgagtgagtttgacatcttcatcaactacatagaagcctacatgacaatgaagatacgaaactgagacatcagggtggcgactctatagactctaggacataaattagaggtctccaaaatcggatctggggctctgggatagctgacccagccccttgagaaaccttattgtacctctcttatagaatatttattacctctgatacctcaacccccatttctatttatttactgagcttctctgtgaacgatttagaaagaagcccaatattataatttttttcaatatttattattttcacctgtttttaagctgtttccatagggtgacacactatggtatttgagtgttttaagataaattataagttacataagggaggaaaaaaaatgttctttggggagccaacagaagcttccattccaagcctgaccacgctttctagctgttgagctgttttccctgacctccctctaatttatcttgtctctgggcttggggcttcctaactgctacaaatactcttaggaagagaaaccagggagcccctttgatgattaattcaccttccagtgtctcggagggattcccctaacctcattccccaaccacttcattcttgaaagctgtggccagcttgttatttataacaacctaaatttggttctaggccgggcgcggtggctcacgcctgtaatcccagcactttgggaggctgaggcgggtggatcacttgaggtcaggagttcctaaccagcctggtcaacatggtgaaaccccgtctctactaaaaatacaaaaattagccgggcatggtggcgcgcacctgtaatcccagctacttgggaggctgaggcaagagaattgcttgaacccaggagatggaagttgcagtgagctgatatcatgcccctgtactccagcctgggtgacagagcaagactctgtctcaaaaaataaaaataaaaataaatttggttctaatagaactcagttttaactagaatttattcaattcctctgggaatgttacattgtttgtctgtcttcatagcagattttaattttgaataaataaatgtatcttattcacatc

SEQ ID NO: 3 - DNA, 537 bp, Artificial Sequence
  codon optimized human IL-10 sequence
atgcacagctcagcactgctgtgctgcctggtcctgctgacaggggtgagggcaagcccaggccagggaacccaatctgagaacagctgcacccacttccctggcaatctgcctaacatgctgcgcgacctccgagatgccttcagcagagtgaagacttttttccagatgaaggatcagctggacaacctgctgctgaaggagtccctcctggaggactttaagggctacctgggatgccaggccctgtctgagatgatccaattctacctggaagaagttatgccccaggctgagaaccaggacccagacattaaggcccatgtcaactccctgggggaaaatctgaagaccctcaggctgcggctacggcgctgtcaccgttttctgccctgtgagaataagagcaaggctgtggagcaggtgaagaacgccttcaataagctccaggagaagggtatctacaaagcgatgagtgaatttgatatcttcattaattatatagaagcttatatgacaatgaaaatcagaaactga

SEQ ID NO: 4 - protein, 185 aa, Homo sapiens
MKLWDVVAVCLVLLHTASAFPLPAANMPEDYPDQFDDVMDFIQATIKRLKRSPDKQMAVLPRRERNRQAAAANPENSRGKGRRGQRGKNRGCVLTAIHLNVTDLGLGYETKEELIFRYCSGSCDAAETTYDKILKNLSRNRRLVSDKVGQACCRPIAFDDDLSFLDDNLVYHILRKHSAKRCGCI

SEQ ID NO: 5 - DNA, 558 bp, Homo sapiens
atgaagttatgggatgtcgtggctgtctgcctggtgctgctccacaccgcgtccgccttcccgctgcccgccgcaaatatgccagaggattatcctgatcagttcgatgatgtcatggattttattcaagccaccattaaaagactgaaaaggtcaccagataaacaaatggcagtgcttcctagaagagagcggaatcggcaggctgcagctgccaacccagagaattccagaggaaaaggtcggagaggccagaggggcaaaaaccggggttgtgtcttaactgcaatacatttaaatgtcactgacttgggtctgggctatgaaaccaaggaggaactgatttttaggtactgcagcggctcttgcgatgcagctgagacaacgtacgacaaaatattgaaaaacttatccagaaatagaaggctggtgagtgacaaagtagggcaggcatgttgcagacccatcgcctttgatgatgacctgtcgtttttagatgataacctggtttaccatattctaagaaagcattccgctaaaaggtgtggatgtatctga

SEQ ID NO: 6 - DNA, 558 bp, Artificial Sequence
  Codon optimized human GDNF DNA
atgaaactttgggacgtggtggctgtctgcctggtgctcctccacaccgccagtgcgtttccgctgcccgccgctaacatgccagaggattatcctgatcagttcgatgatgttatggacttcattcaagccacaatcaagcggctgaaacgatcaccagataaacagatggcagtgcttcctcgccgcgagcgtaatcggcaggctgcagcagccaatcccgagaattcccgaggaaaagggcgcaggggtcagaggggcaagaaccgggggtgtgtcctgactgcaatacatttaaacgtgactgacttgggtctgggctatgagaccaaggaagaactcattttcaggtactgcagcggctcttgcgatgccgcggaaacaacgtacgacaaaatcttgaagaacctctccagaaacagaaggctggtgagtgacaaggtaggacaggcctgttgcagacccatcgcctttgacgacgatctgagctttctggatgacaatctggtttaccacatcctacggaagcattctgctaaaagatgtggatgtatttga

SEQ ID NO: 7 - protein, 585 aa, Homo sapiens
MASPGSGFWSFGSEDGSGDSENPGTARAWCQVAQKFTGGIGNKLCALLYGDAEKPAESGGSQPPRAAARKAACACDQKPCSCSKVDVNYAFLHATDLLPACDGERPTLAFLQDVMNILLQYVVKSFDRSTKVIDFHYPNELLQEYNWELADQPQNLEEILMHCQTTLKYAIKTGHPRYFNQLSTGLDMVGLAADWLTSTANTNMFTYEIAPVFVLLEYVTLKKMREIIGWPGGSGDGIFSPGGAISNMYAMMIARFKMFPEVKEKGMAALPRLIAFTSEHSHFSLKKGAAALGIGTDSVILIKCDERGKMIPSDLERRILEAKQKGFVPFLVSATAGTTVYGAFDPLLAVADICKKYKIWMHVDAAWGGGLLMSRKHKWKLSGVERANSVTWNPHKMMGVPLQCSALLVREEGLMQNCNQMHASYLFQQDKHYDLSYDTGDKALQCGRHVDVFKLWLMWRAKGTTGFEAHVDKCLELAEYLYNIIKNREGYEMVFDGKPQHTNVCFWYIPPSLRTLEDNEERMSRLSKVAPVIKARMMEYGTTMVSYQPLGDKVNFFRMVISNPAATHQDIDFLIEEIERLGQDL

SEQ ID NO: 8 - DNA, 2824 bp, Homo sapiens
gcggccgcccgcacttcccgcctctggctcgcccgaggacgcgctggcacgcctcccaccccctcactctgactccagctggcgtgcatggtctgcctcgcatcctcacgactcagctccctccctctctcgtgtttttttcctccgccgccccctcattcatccccactgggctccctttccctcaaatgctctggggctctccgcgctttcctgagtccgggctccgaggacccttaggtagtcccggtctcttttaaagctccccggcttccaaagggttgccacgtccctaaaccctgtctccagctcgcatacacacacgcacagacacgcacgttttctgttcctgcgtgacacccgccctcgccgctcggccccgccggtccccgcgcggtgccctcctcccgccacacgggcacgcacgcgcgcgcagggccaagcccgaggcagctcgcccgcagctcgcactcgcaggcgacctgctccagtctccaaagccgatggcatctccgggctctggcttttggtctttcgggtcggaagatggctctggggattccgagaatcccggcacagcgcgagcctggtgccaagtggctcagaagttcacgggcggcatcggaaacaaactgtgcgccctgctctacggagacgccgagaagccggcggagagcggcgggagccaacccccgcgggccgccgcccggaaggccgcctgcgcctgcgaccagaagccctgcagctgctccaaagtggatgtcaactacgcgtttctccatgcaacagacctgctgccggcgtgtgatggagaaaggcccactttggcgtttctgcaagatgttatgaacattttacttcagtatgtggtgaaaagtttcgatagatcaaccaaagtgattgatttccattatcctaatgagcttctccaagaatataattgggaattggcagaccaaccacaaaatttggaggaaattttgatgcattgccaaacaactctaaaatatgcaattaaaacagggcatcctagatacttcaatcaactttctactggtttggatatggttggattagcagcagactggctgacatcaacagcaaatactaacatgttcacctatgaaattgctccagtatttgtgcttttggaatatgtcacactaaagaaaatgagagaaatcattggctggccagggggctctggcgatgggatattttctcccggtggcgccatatctaacatgtatgccatgatgatcgcacgctttaagatgttcccagaagtcaaggagaaaggaatggctgctcttcccaggctcattgccttcacgtctgaacatagtcatttttctctcaagaagggagctgcagccttagggattggaacagacagcgtgattctgattaaatgtgatgagagagggaaaatgattccatctgatcttgaaagaaggattcttgaagccaaacagaaagggtttgttcctttcctcgtgagtgccacagctggaaccaccgtgtacggagcatttgaccccctcttagctgtcgctgacatttgcaaaaagtataagatctggatgcatgtggatgcagcttggggtgggggattactgatgtcccgaaaacacaagtggaaactgagtggcgtggagagggccaactctgtgacgtggaatccacacaagatgatgggagtccctttgcagtgctctgctctcctggttagagaagagggattgatgcagaattgcaaccaaatgcatgcctcctacctctttcagcaagataaacattatgacctgtcctatgacactggagacaaggccttacagtgcggacgccacgttgatgtttttaaactatggctgatgtggagggcaaaggggactaccgggtttgaagcgcatgttgataaatgtttggagttggcagagtatttatacaacatcataaaaaaccgagaaggatatgagatggtgtttgatgggaagcctcagcacacaaatgtctgcttctggtacattcctccaagcttgcgtactctggaagacaatgaagagagaatgagtcgcctctcgaaggtggctccagtgattaaagccagaatgatggagtatggaaccacaatggtcagctaccaacccttgggagacaaggtcaatttcttccgcatggtcatctcaaacccagcggcaactcaccaagacattgacttcctgattgaagaaatagaacgccttggacaagatttataataaccttgctcaccaagctgttccacttctctagagaacatgccctcagctaagccccctactgagaaacttcctttgagaattgtgcgacttcacaaaatgcaaggtgaacaccactttgtctctgagaacagacgttaccaattatggagtgtcaccagctgccaaaatcgtaggtgttggctctgctggtcactggagtagttgctactcttcagaatatggacaaagaaggcacaggtgtaaatatagtagcaggatgaggaacctcaaactgggtatcattttgcacgtgctcttctgttctcaaatgctaaatgcaaacactgtgtatttattagttaggtgtgccaaactaccgttcccaaattggtgtttctgaatgacatcaacattcccccaacattactccattactaaagacagaaaaaaataaaaacataaaatatacaaacatgtggcaacctgttcttcctaccaaatataaacttgtgtatgatccaagtattttatctgtgttgtctctctaaacccaaataaatgtgtaaatgtggacacatctc

SEQ ID NO: 9 - protein, 594 aa, Homo sapiens
MASSTPSSSATSSNAGADPNTTNLRPTTYDTWCGVAHGCTRKLGLKICGFLQRTNSLEEKSRLVSAFKERQSSKNLLSCENSDRDARFRRTETDFSNLFARDLLPAKNGEEQTVQFLLEVVDILLNYVRKTFDRSTKVLDFHHPHQLLEGMEGFNLELSDHPESLEQILVDCRDTLKYGVRTGHPRFFNQLSTGLDIIGLAGEWLTSTANTNMFTYEIAPVFVLMEQITLKKMREIVGWSSKDGDGIFSPGGAISNMYSIMAARYKYFPEVKTKGMAAVPKLVLFTSEQSHYSIKKAGAALGFGTDNVILIKCNERGKIIPADFEAKILEAKQKGYVPFYVNATAGTTVYGAFDPIQEIADICEKYNLWLHVDAAWGGGLLMSRKHRHKLNGIERANSVTWNPHKMMGVLLQCSAILVKEKGILQGCNQMCAGYLFQPDKQYDVSYDTGDKAIQCGRHVDIFKFWLMWKAKGTVGFENQINKCLELAEYLYAKIKNREEFEMVFNGEPEHTNVCFWYIPQSLRGVPDSPQRREKLHKVAPKIKALMMESGTTMVGYQPQGDKANFFRMVISNPAATQSDIDFLIEEIERLGQDL

SEQ ID NO: 10 - DNA, 1784 bp, Homo sapiens
atggcgtctcgaccccatcttcgtccgcaacctcctcgaacgcgggagcggaccccaataccactaacctgcgccccacaacgtacgatacctggtgcggcgtggcccatggatgcaccagaaaactggggctcaagatctgcggcttcttgcaaaggaccaacagcctggaagagaagagtcgccttgtgagtgccttcaaggagaggcaatcctccaagaacctgctttcctgtgaaaacagcgaccgggatgcccgcttccggcgcacagagactgacttctctaatctgtttgctagagatctgcttccggctaagaacggtgaggagcaaaccgtgcaattcctcctggaagtggtggacatactcctcaactatgtccgcaagacatttgatcgctccaccaaggtgctggactttcatcacccacaccagttgctggaaggcatggagggcttcaacttggagctctctgaccaccccgagtccctggagcagatcctggttgactgcagagacaccttgaagtatggggttcgcacaggtcatcctcgatttttcaaccagctctccactggattggatattattggcctagctggagaatggctgacatcaacggccaataccaacatgtttacatatgaaattgcaccagtgtttgtcctcatggaacaaataacacttaagaagatgagagagatagttggatggtcaagtaaagatggtgatgggatattttctcctgggggcgccatatccaacatgtacagcatcatggctgctcgctacaagtacttcccggaagttaagacaaagggcatggcggctgtgcctaaactggtcctcttcacctcagaacagagtcactattccataaagaaagctggggctgcacttggctttggaactgacaatgtgattttgataaagtgcaatgaaagggggaaaataattccagctgattttgaggcaaaaattcttgaagccaaacagaagggatatgttcccttttatgtcaatgcaactgctggcacgactgtttatggagcttttgatccgatacaagagattgcagatatatgtgagaaatataacctttggttgcatgtcgatgctgcctggggaggtgggctgctcatgtccaggaagcaccgccataaactcaacggcatagaaagggccaactcagtcacctggaaccctcacaagatgatgggcgtgctgttgcagtgctctgccattctcgtcaaggaaaagggtatactccaaggatgcaaccagatgtgtgcaggatacctcttccagccagacaagcagtatgatgtctcctacgacaccggggacaaggcaattcagtgtggccgccacgtggatatcttcaagttctggctgatgtggaaagcaaagggcacagtgggatttgaaaaccagatcaacaaatgcctggaactggctgaatacctctatgccaagattaaaaacagagaagaatttgagatggttttcaatggcgagcctgagcacacaaacgtctgtttttggtatattccacaaagcctcaggggtgtgccagacagccctcaacgacgggaaaagctacacaaggtggctccaaaaatcaaagccctgatgatggagtcaggtacgaccatggttggctaccagccccaaggggacaaggccaacttcttccggatggtcatctccaacccagccgctacccagtctgacattgacttcctcattgaggagatagaaagactgggccaggatctgtaa

SEQ ID NO: 11 - DNA, 28 bp, Artificial Sequence
  Forward primer for amplifying CMV promoter(F-JDK)
ttcggccgtcgaggagcttggcccattg

SEQ ID NO: 12 - DNA, 36 bp, Artificial Sequence
  Reverse primer for amplifying CMV promoter(R-JDK)
gacgtcgacctagctagcgaattcggggccgcggag

SEQ ID NO: 13 - DNA, 34 bp, Artificial Sequence
  Forward primer for amplifying SV40pA promoter(F-SV40pA)
ccatcgatcagacatgataagatacattgatgag

SEQ ID NO: 14 - DNA, 43 bp, Artificial Sequence
  Reverse primer for amplifying SV40pA promoter(R-SV40pA)
gacgtcgacgcggccgctaccacatttgtagaggttttacttg

SEQ ID NO: 15 - DNA, 43 bp, Artificial Sequence
  Forward primer for SV40-CMV-sCAG-bGHpA-Infu-F
cctgcggccggtcgactaccacatttgtagaggttttacttgc

SEQ ID NO: 16 - DNA, 35 bp, Artificial Sequence
  Reverse primer for SV40-CMV-sCAG-bGHpA-Infu-R
aataatcaatgtcgactcgaggagcttggcccatt